European Patent Application EP 4 606 903 A1, published August 27, 2025. Title: Method for Enzymatic Synthesis of Nucleoside Bearing Protecting Group, and Composition. Applicant: Asymchem Life Science (Tianjin) Co., Ltd. The sequence listing filed with the application follows.

SEQUENCE LISTING (8 sequences)

SEQ ID NO: 1 - protein, 423 aa, Thermus thermophilus
MNPVAFIREKREGKKHRREDLEAFLLGYLRDEVPDYQVSAWLMAAFLRGLDPEETLWLTETMARSGKVLDLSGLPHPVDKHSSGGVGDKVSLVVGPILAASGCTFAKMSGRGLAHTGGTIDKLESVPGWRGEMTEAEFLERARRVGLVIAAQSPDLAPLDGKLYALRDVTATVESVPLIASSIMSKKLAAGARSIVLDVKVGRGAFMKTLEEARLLAKTMVAIGQGAGRRVRALLTSMEAPLGRAVGNAIEVREAIEALKGEGPGDLLEVALALAEEALRLEGLDPALARKALEGGAALEKFRAFLEAQGGDPRAVEDFSLLPLAEEHPLRAEREGVVREVDAYKVGLAVLALGGGRKRKGEPIDHGVGVYLLKKPGDRVERGEALALVYHRRRGLEEALGHLREAYALGEEAHPAPLVLEAI

SEQ ID NO: 2 - protein, 344 aa, Trypanosoma cruzi
MSKATHTHGLMKDPDLPVTADGVTYHLNCKSDQLADRILLVGDPGRVDTVAACFDAGSVRFRSENREIFIATGTYKGTPVSVLSTGMGTDNVEIVINEIHLLKEYDFERCSWRPRVGDADVPPGAKVFDPSSVKMIRVGTCGSPFPDMPLAALAITRHVIGMDNTCLYYKVKEQMQKSKDLQEVQRVVKEQTSLGAIDVYATKAHPAITNGIVAACKAFNDNLPAGATEQLYVVGATATASGFYACQGRAVGRFREHLLVPKLVEELSKVQFDVSEGKEIVANIEMETSAVCFLSHLLGYQAGSMCVVVAKRAGAEHLFTTSEQSGQALKNAIQIALEAIVAVG

SEQ ID NO: 3 - protein, 235 aa, Geobacillus thermoglucosidasius
MSIHIEAKQQEIAEKILLPGDPLRAQYIAETFLEGATCYNRVRGMLGFTGTYKGHRISVQGTGMGVPSISIYVNELIQSYHVQTLIRVGTCGAIQKDVNVRDVILAMSASTDSNMNRLTFRGRDYAPTANFALLRTAYEVGAEKGLPLKVGSVFTADMFYNDEPDWETWARYGVLAVEMETAALYTLAAKFGRKALSVLTVSDHILTGEETTAQERQTTFNDMIEVALETAIRVE

SEQ ID NO: 4 - DNA, 1272 bp, synthetic construct
  source 1..1272: mol_type = other DNA; note = DNA sequence of PyNP
atgaacccggtggcgtttattcgcgaaaaacgcgaaggcaagaaacatcgccgcgaggatctggaagcgtttctgctgggctatctgcgcgatgaagtgccggattatcaggtgagcgcgtggctgatggcggcgtttttacgcggcttagatccggaagaaaccctgtggctgaccgaaacgatggcccgcagcggtaaagtgctggatctgagcggtctgccgcatccggttgataaacatagcagcggcggcgtgggcgataaagtgagcttagtggtgggcccgattctggcggcgagcggttgtacctttgcgaaaatgtcgggccgcggcctggcgcataccggtggtaccattgataaactggaaagcgtgccgggctggcgcggcgaaatgaccgaagcagaatttctggaacgcgcccgtcgcgttggtctggttattgcggcgcaaagcccggatttagcgccgttagatggcaaactgtatgcgctgcgcgatgtgaccgcgaccgttgaatcagttccgctgattgcgagcagcattatgagcaagaaactggcggcgggcgcccgtagcattgtgttagatgttaaagtgggccgcggcgcgtttatgaaaaccctggaagaagcgcgtctgctggcgaaaacgatggtggcgattggccagggcgcgggccgtcgtgttcgtgcgttattaaccagcatggaagcgcctctgggtcgtgcggttggcaatgcgattgaagtgcgtgaagcgattgaagcgctgaaaggcgaaggcccgggcgatttattagaagtggcgctggcgttagcggaagaagcgctgcgtttagaaggcttagatccggcgctggcgcgtaaagcgttagaaggtggcgcggcgctggaaaaatttcgcgcgtttctggaagcgcagggcggcgatccgcgtgcagttgaagattttagcctgctgccgctggcggaagaacatccgttacgtgcggaacgcgaaggcgtggttcgcgaagttgatgcgtataaagtgggcctggcggtgctggcgttaggcggtggtcgtaaacgtaaaggtgaaccgattgatcatggcgtgggcgtgtatctgctgaagaaaccgggcgatcgcgtggaacgcggcgaagcgttagcgttagtgtatcatcgccgccgcggcttagaagaagcgctgggtcatttacgcgaagcgtatgcgctgggcgaagaagcgcatccggcgcctctggttttagaagcgatttaa

SEQ ID NO: 5 - DNA, 1035 bp, synthetic construct
  source 1..1035: mol_type = other DNA; note = DNA sequence of UP
atgagcaaagcgacccatacccacggcctgatgaaagatccggatctgccggtgacggcggatggcgttacctatcatctgaactgcaaaagcgatcagctggcggatcgcattctgctggtgggcgatccgggtcgcgttgataccgtagcggcatgttttgatgcgggcagcgttcgctttcgcagcgaaaaccgcgaaatttttattgcgaccggcacctataaaggcaccccggtgtcagtgctgagcaccggtatgggtactgataatgtggaaattgtgattaacgagattcacctgctgaaggagtatgacttcgagcgctgcagctggcgcccgcgtgttggtgatgcggatgttcctcctggtgcgaaagtgtttgatccgagcagcgtgaaaatgattcgcgtgggcacctgcggcagcccgtttcctgatatgcctctggcggcgctggcgattacccgccatgttattggcatggataacacctgcctgtattataaagtgaaagagcagatgcagaagagcaaggatctgcaggaagtgcagcgcgtggtgaaagaacagaccagcctgggcgcgattgatgtgtatgcgaccaaagcgcatccggcgattaccaacggcattgtggcggcgtgtaaagcgtttaacgataacctgccggcgggcgcgactgaacaattatatgttgttggcgcgaccgcgaccgcgagcggtttttatgcgtgtcaaggtcgcgcggtgggccgctttcgtgaacatttactggttccgaaactggtggaagaactgagcaaagtgcagtttgatgtgagcgaaggcaaagaaattgtggcgaacattgaaatggaaaccagcgcggtgtgctttctgagccatctgctgggctatcaggcgggctcaatgtgcgttgttgttgcgaaacgcgcgggcgcggaacatctgtttaccaccagcgaacagagcggccaggcgctgaaaaacgcgattcagattgcgctggaagcgattgtggcggtgggctaa

SEQ ID NO: 6 - DNA, 708 bp, synthetic construct
  source 1..708: mol_type = other DNA; note = DNA sequence of PNP
atgagcattcatattgaagcgaaacagcaggaaattgcggaaaagattctgctgccgggcgatccgttacgtgcgcaatatattgcggaaacctttctggaaggcgcgacctgctataaccgcgtgcgcggtatgctgggctttaccggtacctataaaggccatcgcattagcgtgcagggcaccggcatgggcgttccgtcaattagcatttatgtgaacgaactgattcagagctatcacgtgcagaccctgattcgcgtgggcacctgtggcgcaattcagaaagatgtgaacgtgcgcgatgtgattctggcgatgagcgcgagcaccgatagcaacatgaaccgcctgacctttcgcggccgtgattatgcgcctaccgcgaattttgcgctgctgcgcactgcgtatgaagtgggcgcggaaaaaggcctgccgctgaaagtgggcagcgtgtttaccgcggatatgttttataacgatgaaccggattgggaaacctgggcccgctatggcgttctggcggtggaaatggaaaccgcggcgttatataccctggcggcgaaatttggccgcaaagcgctgagcgtgctgaccgtgagcgatcatattctgaccggcgaagaaaccaccgcgcaggaacgccaaaccacctttaacgatatgattgaagtggcgctggaaaccgcgattcgcgtggaataa

SEQ ID NO: 7 - protein, 275 aa, Thermus thermophilus
MPGMELYDKIQEAVAYVRSKTDFVPEVGLVLGSGLGPLADEVEKVAEIPYGEIPHFPVSTAPGHAGRLVLGRLEGKPVLVYKGRVHYYEGYSAEEVVFPVRVGFFLGARTFLLTSAAGGLNPRFRAGGIMLHLDYINFAGANPLRGPNDERLGPRFPVMFEAYDPELIELARKVARRQDLHLFEGVYAWFMGPSFASRAELKLLRELGADAIGMSTVPEVIALRHLGARVLGLSTITDMAVPEREHHATEEEVLRVAAETGPVFRRYVRGILAEL

SEQ ID NO: 8 - protein, 261 aa, Deinococcus geothermalis
MVARVPARPFASPPATLDRVSVHLNARPGEIAETVLLPGDPLRAQHIAETFFENPVQHNSVRGMLGFTGTYRGVPVSVQGTGMGIASSMIYVNELIRDYGCQTLIRVGTAGSYQPDVHVRDLVLAQAACTDSNINNIRFGLRNFAPIADFELLLRAYQMARDRGFATHVGNILSSDTFYQDDPESYKLWAQYGVLAVEMEAAGLYTLAAKYGVRALTILTISDHLVTREETTAEERQTTFNGMIEVALDAALGLAVPSNSM